European Patent Application EP 4 119 675 A1, published January 18, 2023. Title: METHODS FOR DETECTING GENE DYSREGULATIONS. Applicant: QUEST DIAGNOSTICS INVESTMENTS INCORPORATED. Application Divisional application based on EP 19151537.8. The sequence listing filed with the application follows.

SEQUENCE LISTING (18 sequences)

SEQ ID NO: 1 - DNA, 20 bp, Artificial Sequence
  Description of Artificial Sequence: Synthetic primer
taggcgcgagctaagcagga

SEQ ID NO: 2 - DNA, 19 bp, Artificial Sequence
  Description of Artificial Sequence: Synthetic primer
cctgccgcgctccaggcgg

SEQ ID NO: 3 - DNA, 24 bp, Artificial Sequence
  Description of Artificial Sequence: Synthetic probe
aggcggaggcggagggcgaggggc

SEQ ID NO: 4 - DNA, 18 bp, Artificial Sequence
  Description of Artificial Sequence: Synthetic primer
tggtgcgagggaagcaat

SEQ ID NO: 5 - DNA, 19 bp, Artificial Sequence
  Description of Artificial Sequence: Synthetic primer
cacccaatgtgcaggtgga

SEQ ID NO: 6 - DNA, 24 bp, Artificial Sequence
  Description of Artificial Sequence: Synthetic probe
aaaggaacttgccctgagcactcc

SEQ ID NO: 7 - DNA, 21 bp, Artificial Sequence
  Description of Artificial Sequence: Synthetic primer
catccgctctaaacaacctca

SEQ ID NO: 8 - DNA, 20 bp, Artificial Sequence
  Description of Artificial Sequence: Synthetic primer
ggccataatgcgatcaagtt

SEQ ID NO: 9 - DNA, 22 bp, Artificial Sequence
  Description of Artificial Sequence: Synthetic probe
ctttctggtcagagagaagcaa

SEQ ID NO: 10 - DNA, 21 bp, Artificial Sequence
  Description of Artificial Sequence: Synthetic primer
ccaggtgaatggctcaaggaa

SEQ ID NO: 11 - DNA, 18 bp, Artificial Sequence
  Description of Artificial Sequence: Synthetic primer
gggctgcccaccatcttc

SEQ ID NO: 12 - DNA, 24 bp, Artificial Sequence
  Description of Artificial Sequence: Synthetic probe
tctcctgatgaatgcagtgtggcc

SEQ ID NO: 13 - DNA, 20 bp, Artificial Sequence
  Description of Artificial Sequence: Synthetic primer
cccaactttgccatcatttt

SEQ ID NO: 14 - DNA, 20 bp, Artificial Sequence
  Description of Artificial Sequence: Synthetic primer
gcaaagcggtgttgattaca

SEQ ID NO: 15 - DNA, 20 bp, Artificial Sequence
  Description of Artificial Sequence: Synthetic probe
tgaatactgcacccaggacc

SEQ ID NO: 16 - DNA, 21 bp, Artificial Sequence
  Description of Artificial Sequence: Synthetic primer
tggcttttgacaatatctcca

SEQ ID NO: 17 - DNA, 20 bp, Artificial Sequence
  Description of Artificial Sequence: Synthetic primer
tgcaggatcttgtcctctcc

SEQ ID NO: 18 - DNA, 20 bp, Artificial Sequence
  Description of Artificial Sequence: Synthetic probe
agcctggactgctacctcac